European Patent Specification EP 3 604 345 B1, published May 10, 2023. Title: ANTI-TUMOR PEPTIDES AND USE THEREOF. Applicant: TOAGOSEI CO., LTD NAGOYA UNIVERSITY. The sequence listing filed with the application follows.

SEQUENCE LISTING (30 sequences)

SEQ ID NO: 1 - protein, 20 aa, Artificial Sequence
  Synthetic peptide
MQIPQAPWPVVWAVLQLGWR

SEQ ID NO: 2 - protein, 20 aa, Artificial Sequence
  Synthetic peptide
MWVRQVPWSFTWAVLQLSWQ

SEQ ID NO: 3 - protein, 29 aa, Artificial Sequence
  Synthetic peptide
MGTPRALWPLVWAVLQLGCWPGWLLEASS

SEQ ID NO: 4 - protein, 29 aa, Artificial Sequence
  Synthetic peptide
MGTPRALWPLVWAVLQLGCWPGWLLEASS

SEQ ID NO: 5 - protein, 24 aa, Artificial Sequence
  Synthetic peptide
MGTPRAPWPLVWAVLQLGWWPGWL

SEQ ID NO: 6 - protein, 20 aa, Artificial Sequence
  Synthetic peptide
MQIPQAPWPVVWAVLQLGWR

SEQ ID NO: 7 - protein, 20 aa, Artificial Sequence
  Synthetic peptide
MWVQQVPWSFTWAVLQLSWQ

SEQ ID NO: 8 - protein, 14 aa, Artificial sequence
  Synthetic peptide
RSRKYTSWYVALKR

SEQ ID NO: 9 - protein, 19 aa, Artificial sequence
  Synthetic peptide
MAKSIRSKHRRQMRMMKRE

SEQ ID NO: 10 - protein, 16 aa, Artificial sequence
  Synthetic peptide
MARRRRHRGPRRPRPP

SEQ ID NO: 11 - protein, 19 aa, Artificial sequence
  Synthetic peptide
GRCRRLANFGPRKRRRRRR

SEQ ID NO: 12 - protein, 16 aa, Artificial sequence
  Synthetic peptide
RRRKRNRDARRRRRKQ

SEQ ID NO: 13 - protein, 17 aa, Artificial sequence
  Synthetic peptide
MQRKPTIRRKNLRLRRK

SEQ ID NO: 14 - protein, 7 aa, Artificial sequence
  Synthetic peptide
IMRRRGL

SEQ ID NO: 15 - protein, 8 aa, Artificial sequence
  Synthetic peptide
KKLKKRNK

SEQ ID NO: 16 - protein, 9 aa, Artificial sequence
  Synthetic peptide
RRRANNRRR

SEQ ID NO: 17 - protein, 7 aa, Artificial sequence
  Synthetic peptide
RKKRKKK

SEQ ID NO: 18 - protein, 15 aa, Artificial sequence
  Synthetic peptide
KRKGKLKNKGSKRKK

SEQ ID NO: 19 - protein, 18 aa, Artificial sequence
  Synthetic peptide
SKRLSSRARKRAAKRRLG

SEQ ID NO: 20 - protein, 14 aa, Artificial sequence
  Synthetic peptide
KRPRRRPSRPFRKP

SEQ ID NO: 21 - protein, 13 aa, Artificial sequence
  Synthetic peptide
KKRTLRKNDRKKR

SEQ ID NO: 22 - protein, 8 aa, Artificial Sequence
  Synthetic peptide
WRRQARFK

SEQ ID NO: 23 - protein, 9 aa, Artificial Sequence
  Synthetic peptide
RKKRRQRRR

SEQ ID NO: 24 - protein, 11 aa, Artificial Sequence
  Synthetic peptide
YARAAARQARA

SEQ ID NO: 25 - protein, 18 aa, Artificial Sequence
  Synthetic peptide
KGRQVKVWFQNRRMKWKK

SEQ ID NO: 26 - protein, 33 aa, Artificial Sequence
  Synthetic peptide
MQIPQAPWPVVWAVLQLGWRKKRTLRKNDRKKR

SEQ ID NO: 27 - protein, 29 aa, Artificial Sequence
  Synthetic peptide
MQIPQAPWPVVWAVLQLGWRRKKRRQRRR

SEQ ID NO: 28 - protein, 31 aa, Artificial Sequence
  Synthetic peptide
MRIFAVFIFMTYWHLLNAKKRTLRKNDRKKR

SEQ ID NO: 29 - protein, 33 aa, Artificial Sequence
  Synthetic peptide
PWWWPPVVVQQQMLLIGAARKKRTLRKNDRKKR

SEQ ID NO: 30 - protein, 13 aa, Artificial Sequence
  Synthetic peptide
KKRTLRKNDRKKR